European Patent Specification EP 3 755 357 B1, published September 17, 2025. Title: Pathogenic Bacteria. Applicant: Sporegen Limited. The sequence listing filed with the application follows.

SEQUENCE LISTING (17 sequences)

SEQ ID NO: 1 - protein, 7 aa, Artificial Sequence
  Iturin A
  MISC_FEATURE (2)..(2): D-Tyr
  MISC_FEATURE (3)..(3): D-Asn
  MISC_FEATURE (6)..(6): D-Asn
NXXQPXS

SEQ ID NO: 2 - protein, 7 aa, Artificial Sequence
  Iturin AL
  MISC_FEATURE (2)..(2): D-Tyr
  MISC_FEATURE (3)..(3): D-Asn
  MISC_FEATURE (6)..(6): D-Asn
NXXQPXS

SEQ ID NO: 3 - protein, 7 aa, Artificial Sequence
  Iturin C
  MISC_FEATURE (2)..(2): D-Tyr
  MISC_FEATURE (3)..(3): D-Asn
  MISC_FEATURE (6)..(6): D-Asn
NXXQPXS

SEQ ID NO: 4 - protein, 7 aa, Artificial Sequence
  Mycosubtilin
  MISC_FEATURE (2)..(2): D-Tyr
  MISC_FEATURE (3)..(3): D-Asn
  MISC_FEATURE (6)..(3): D-Ser
  misc_feature (6)..(6): Xaa can be any naturally occurring amino acid
NXXQPXN

SEQ ID NO: 5 - protein, 7 aa, Artificial Sequence
  Bacillomycin D
  MISC_FEATURE (2)..(2): D-Tyr
  MISC_FEATURE (3)..(3): D-Asn
  MISC_FEATURE (6)..(6): D-Ser
NXXPEXT

SEQ ID NO: 6 - protein, 7 aa, Artificial Sequence
  Bacillomycin F
  MISC_FEATURE (2)..(2): D-Tyr
  MISC_FEATURE (3)..(3): D-Asn
  MISC_FEATURE (6)..(6): D-Asn
NXXQPXT

SEQ ID NO: 7 - protein, 7 aa, Artificial Sequence
  Bacillomycin L
  MISC_FEATURE (2)..(2): D-Tyr
  MISC_FEATURE (3)..(3): D-Asn
  MISC_FEATURE (6)..(6): D-Asn
NXXSQXT

SEQ ID NO: 8 - protein, 7 aa, Artificial Sequence
  Bacillomycin LC
  MISC_FEATURE (2)..(2): D-Tyr
  MISC_FEATURE (3)..(3): D-Asn
  MISC_FEATURE (6)..(6): D-Ser
NXXSQXT

SEQ ID NO: 9 - protein, 7 aa, Artificial Sequence
  Esperin
  MISC_FEATURE (3)..(3): D-Leu
  MISC_FEATURE (6)..(6): D-Leu
ELXVDXL

SEQ ID NO: 10 - protein, 7 aa, Artificial Sequence
  Lichenysin
  MISC_FEATURE (1)..(1): Glu or Gln
  MISC_FEATURE (2)..(2): Leu or Ile
  MISC_FEATURE (3)..(3): D-Leu
  MISC_FEATURE (4)..(4): Val or Ile
  MISC_FEATURE (6)..(6): D-Leu
  MISC_FEATURE (7)..(7): Val or Ile
XXXXDXX

SEQ ID NO: 11 - protein, 7 aa, Artificial Sequence
  Pumilacidin
  MISC_FEATURE (3)..(3): D-Leu
  MISC_FEATURE (6)..(6): D-Leu
  MISC_FEATURE (7)..(7): Val or Ile
ELXLDXX

SEQ ID NO: 12 - protein, 7 aa, Artificial Sequence
  Surfactin
  MISC_FEATURE (2)..(2): Val, Leu or Ile
  MISC_FEATURE (3)..(3): D-leu
  MISC_FEATURE (4)..(4): Ala, Val, Leu or Ile
  MISC_FEATURE (6)..(6): D-Leu
  MISC_FEATURE (7)..(7): Val, Leu or Ile
EXXXDXX

SEQ ID NO: 13 - protein, 10 aa, Artificial Sequence
  Fengycin A
  MISC_FEATURE (2)..(2): Orn
  MISC_FEATURE (3)..(3): D-Tyr
  MISC_FEATURE (4)..(4): aThr
  MISC_FEATURE (6)..(6): D-Ala
  MISC_FEATURE (9)..(9): D-Ala
EXXXEXPQTI

SEQ ID NO: 14 - protein, 10 aa, Artificial Sequence
  Fengycin B
  MISC_FEATURE (2)..(2): D-Orn
  MISC_FEATURE (3)..(3): D-Tyr
  MISC_FEATURE (4)..(4): D-aThr
  MISC_FEATURE (6)..(6): D-Val
EXXXEXPQTI

SEQ ID NO: 15 - protein, 10 aa, Artificial Sequence
  Plipastatin A
  MISC_FEATURE (2)..(2): D-Orn
  MISC_FEATURE (4)..(4): D-aThr
  MISC_FEATURE (6)..(6): D-Ala
  MISC_FEATURE (9)..(9): D-Tyr
EXTXEXPQXI

SEQ ID NO: 16 - protein, 10 aa, Artificial Sequence
  Plipastatin B
  MISC_FEATURE (2)..(2): D-Orn
  MISC_FEATURE (4)..(4): D-aThr
  MISC_FEATURE (6)..(6): D-Ala
  MISC_FEATURE (9)..(9): D-Tyr
EXTXEXPQXI

SEQ ID NO: 17 - protein, 8 aa, Artificial Sequence
  Bacillopeptin
  MISC_FEATURE (1)..(1): D-Asn
  MISC_FEATURE (4)..(4): D-Ser
  MISC_FEATURE (6)..(6): Beta amino acid
  MISC_FEATURE (8)..(8): D-Tyr
XSEXTXNX